European Patent Application EP 4 163 382 A1, published April 12, 2023. Title: Phagemid Vector. Applicant: Imperial College Innovations Limited. Application GB PCT/GB2016/053366, filed October 31, 2016. The sequence listing filed with the application follows.

SEQUENCE LISTING (13 sequences)

SEQ ID NO: 1 - DNA, 456 bp, unidentified
  source 1..456: mol_type = unassigned DNA; note = DNA sequence of an F1 bacteriophage ori
acgcgccctgtagcggcgcattaagcgcggcgggtgtggtggttacgcgcagcgtgaccgctacacttgccagcgccctagcgcccgctcctttcgctttcttcccttcctttctcgccacgttcgccggctttccccgtcaagctctaaatcgggggctccctttagggttccgatttagtgctttacggcacctcgaccccaaaaaacttgatttgggtgatggttcacgtagtgggccatcgccctgatagacggtttttcgccctttgacgttggagtccacgttctttaatagtggactcttgttccaaactggaacaacactcaaccctatctcgggctattcttttgatttataagggattttgccgatttcggcctattggttaaaaaatgagctgatttaacaaaaatttaacgcgaattttaacaaaatattaacgtttacaattt

SEQ ID NO: 2 - DNA, 589 bp, unidentified
  source 1..589: mol_type = unassigned DNA; note = DNA sequence of a PUC ori of an origin of replication
ttgagatcctttttttctgcgcgtaatctgctgcttgcaaacaaaaaaaccaccgctaccagcggtggtttgtttgccggatcaagagctaccaactctttttccgaaggtaactggcttcagcagagcgcagataccaaatactgtccttctagtgtagccgtagttaggccaccacttcaagaactctgtagcaccgcctacatacctcgctctgctaatcctgttaccagtggctgctgccagtggcgataagtcgtgtcttaccgggttggactcaagacgatagttaccggataaggcgcagcggtcgggctgaacggggggttcgtgcacacagcccagcttggagcgaacgacctacaccgaactgagatacctacagcgtgagctatgagaaagcgccacgcttcccgaagggagaaaggcggacaggtatccggtaagcggcagggtcggaacaggagagcgcacgagggagcttccagggggaaacgcctggtatctttatagtcctgtcgggtttcgccacctctgacttgagcgtcgatttttgtgatgctcgtcaggggggcggagcctatggaaa

SEQ ID NO: 3 - DNA, 663 bp, unidentified
  source 1..663: mol_type = unassigned DNA; note = A DNA sequence of a promoter of a Cytomegalovirus
acgcgtggagctagttattaatagtaatcaattacggggtcattagttcatagcccatatatggagttccgcgttacataacttacggtaaatggcccgcctggctgaccgcccaacgacccccgcccattgacgtcaataatgacgtatgttcccatagtaacgtcaatagggactttccattgacgtcaatgggtggagtatttacggtaaactgcccacttggcagtacatcaagtgtatcatatgccaagtacgccccctattgacgtcaatgacggtaaatggcccgcctggcattatgcccagtacatgaccttatgggactttcctacttggcagtacatctacgtattagtcatcgctattaccatggtgatgcggttttggcagtacatcaatgggcgtggatagcggtttgactcacggggatttccaagtctccaccccattgacgtcaatgggagtttgttttgcaccaaaatcaacgggactttccaaaatgtcgtaacaactccgccccattgacgcaaatgggcggtaggcgtgtacggtgggaggtctatataagcagagctcgtttagtgaaccgtcagatcgcctggagacgccatccacgctgttttgacctccatagaagacaccgggaccgatccagcctcc

SEQ ID NO: 4 - DNA, 479 bp, unidentified
  source 1..479: mol_type = unassigned DNA; note = The DNA sequence of one embodiment of a nucleic acid for encoding a polyA tail
acgggtggcatccctgtgacccctccccagtgcctctcctggccctggaagttgccactccagtgcccaccagccttgtcctaataaaattaagttgcatcattttgtctgactaggtgtccttctataatattatggggtggaggggggtggtatggagcaaggggcaagttgggaagacaacctgtagggcctgcggggtctattgggaaccaagctggagtgcagtggcacaatcttggctcactgcaatctccgcctcctgggttcaagcgattctcctgcctcagcctcccgagttgttgggattccaggcatgcatgaccaggctcagctaatttttgtttttttggtagagacggggtttcaccatattggccaggctggtctccaactcctaatctcaggtgatctacccaccttggcctcccaaattgctgggattacaggcgtgaaccactgctcccttccctgtcctt

SEQ ID NO: 5 - DNA, 130 bp, unidentified
  source 1..130: mol_type = unassigned DNA; note = The DNA sequence of one (left) embodiment of an Inverted Terminal Repeat sequences (ITR)
cctgcaggcagctgcgcgctcgctcgctcactgaggccgcccgggcgtcgggcgacctttggtcgcccggcctcagtgagcgagcgagcgcgcagagagggagtggccaactccatcactaggggttcct

SEQ ID NO: 6 - DNA, 141 bp, unidentified
  source 1..141: mol_type = unassigned DNA; note = The DNA sequence of one (right) embodiment of an Inverted Terminal Repeat sequences (ITR)
aggaacccctagtgatggagttggccactccctctctgcgcgctcgctcgctcactgaggccgggcgaccaaaggtcgcccgacgcccgggctttgcccgggcggcctcagtgagcgagcgagcgcgcagctgcctgcagg

SEQ ID NO: 7 - protein, 9 aa, unidentified
  SOURCE 1..9: NOTE = The amino acid sequence of a RGD4C targeting peptide
CDCRGDCFC

SEQ ID NO: 8 - DNA, 378 bp, unidentified
  source 1..378: mol_type = unassigned DNA; note = The nucleic acid sequence of one embodiment of a grp78 promoter
cccgggggcccaacgtgaggggaggacctggacggttaccggcggaaacggtttccaggtgagaggtcacccgagggacaggcagctgctcaaccaataggaccagctctcagggcggatgctgcctctcattggcggccgttaagaatgaccagtagccaatgagtcggctggggggcgcgtaccagtgacgtgagttgcggaggaggccgcttcgaatcggcagcggccagcttggtggcatgaaccaaccagcggcctccaacgagtagcgagttcaccaatcggaggcctccacgacggggctgcggggaggatatataagccgagtcggcgaccggcgcgctcgatactggctgtgactacactgacttggac

SEQ ID NO: 9 - DNA, 2876 bp, unidentified
  source 1..2876: mol_type = unassigned DNA; note = The nucleic acid sequence of one embodiment of a first vector (i.e. a phagemid particle genome)
cctgcaggcagctgcgcgctcgctcgctcactgaggccgcccgggcgtcgggcgacctttggtcgcccggcctcagtgagcgagcgagcgcgcagagagggagtggccaactccatcactaggggttcctgcggccgcaggaacccctagtgatggagttggccactccctctctgcgcgctcgctcgctcactgaggccgggcgaccaaaggtcgcccgacgcccgggctttgcccgggcggcctcagtgagcgagcgagcgcgcagctgcctgcaggggcgcctgatgcggtattttctccttacgcatctgtgcggtatttcacaccgcatacgtcaaagcaaccatagtacgcgccctgtagcggcgcattaagcgcggcgggtgtggtggttacgcgcagcgtgaccgctacacttgccagcgccctagcgcccgctcctttcgctttcttcccttcctttctcgccacgttcgccggctttccccgtcaagctctaaatcgggggctccctttagggttccgatttagtgctttacggcacctcgaccccaaaaaacttgatttgggtgatggttcacgtagtgggccatcgccctgatagacggtttttcgccctttgacgttggagtccacgttctttaatagtggactcttgttccaaactggaacaacactcaaccctatctcgggctattcttttgatttataagggattttgccgatttcggcctattggttaaaaaatgagctgatttaacaaaaatttaacgcgaattttaacaaaatattaacgtttacaattttatggtgcactctcagtacaatctgctctgatgccgcatagttaagccagccccgacacccgccaacacccgctgacgcgccctgacgggcttgtctgctcccggcatccgcttacagacaagctgtgaccgtctccgggagctgcatgtgtcagaggttttcaccgtcatcaccgaaacgcgcgagacgaaagggcctcgtgatacgcctatttttataggttaatgtcatgataataatggtttcttagacgtcaggtggcacttttcggggaaatgtgcgcggaacccctatttgtttatttttctaaatacattcaaatatgtatccgctcatgagacaataaccctgataaatgcttcaataatattgaaaaaggaagagtatgagtattcaacatttccgtgtcgcccttattcccttttttgcggcattttgccttcctgtttttgctcacccagaaacgctggtgaaagtaaaagatgctgaagatcagttgggtgcacgagtgggttacatcgaactggatctcaacagcggtaagatccttgagagttttcgccccgaagaacgttttccaatgatgagcacttttaaagttctgctatgtggcgcggtattatcccgtattgacgccgggcaagagcaactcggtcgccgcatacactattctcagaatgacttggttgagtactcaccagtcacagaaaagcatcttacggatggcatgacagtaagagaattatgcagtgctgccataaccatgagtgataacactgcggccaacttacttctgacaacgatcggaggaccgaaggagctaaccgcttttttgcacaacatgggggatcatgtaactcgccttgatcgttgggaaccggagctgaatgaagccataccaaacgacgagcgtgacaccacgatgcctgtagcaatggcaacaacgttgcgcaaactattaactggcgaactacttactctagcttcccggcaacaattaatagactggatggaggcggataaagttgcaggaccacttctgcgctcggcccttccggctggctggtttattgctgataaatctggagccggtgagcgtgggtctcgcggtatcattgcagcactggggccagatggtaagccctcccgtatcgtagttatctacacgacggggagtcaggcaactatggatgaacgaaatagacagatcgctgagataggtgcctcactgattaagcattggtaactgtcagaccaagtttactcatatatactttagattgatttaaaacttcatttttaatttaaaaggatctaggtgaagatcctttttgataatctcatgaccaaaatcccttaacgtgagttttcgttccactgagcgtcagaccccgtagaaaagatcaaaggatcttcttgagatcctttttttctgcgcgtaatctgctgcttgcaaacaaaaaaaccaccgctaccagcggtggtttgtttgccggatcaagagctaccaactctttttccgaaggtaactggcttcagcagagcgcagataccaaatactgtccttctagtgtagccgtagttaggccaccacttcaagaactctgtagcaccgcctacatacctcgctctgctaatcctgttaccagtggctgctgccagtggcgataagtcgtgtcttaccgggttggactcaagacgatagttaccggataaggcgcagcggtcgggctgaacggggggttcgtgcacacagcccagcttggagcgaacgacctacaccgaactgagatacctacagcgtgagctatgagaaagcgccacgcttcccgaagggagaaaggcggacaggtatccggtaagcggcagggtcggaacaggagagcgcacgagggagcttccagggggaaacgcctggtatctttatagtcctgtcgggtttcgccacctctgacttgagcgtcgatttttgtgatgctcgtcaggggggcggagcctatggaaaaacgccagcaacgcggcctttttacggttcctggccttttgctggccttttgctcacatgt

SEQ ID NO: 10 - DNA, 8696 bp, unidentified
  source 1..8696: mol_type = unassigned DNA; note = The nucleic acid sequence of one embodiment of a second vector (i.e. a helper phage with a RGD sequence)
aacgctactactattagtagaattgatgccaccttttcagctcgcgccccaaatgaaaatatagctaaacaggttattgaccatttgcgaaatgtatctaatggtcaaactaaatctactcgttcgcagaattgggaatcaactgttacatggaatgaaacttccagacaccgtactttagttgcatatttaaaacatgttgagctacagcaccagattcagcaattaagctctaagccatccgcaaaaatgacctcttatcaaaaggagcaattaaaggtactctctaatcctgacctgttggagtttgcttccggtctggttcgctttgaagctcgaattaaaacgcgatatttgaagtctttcgggcttcctcttaatctttttgatgcaatccgctttgcttctgactataatagtcagggtaaagacctgatttttgatttatggtcattctcgttttctgaactgtttaaagcatttgagggggattcaatgaatatttatgacgattccgcagtattggacgctatccagtctaaacattttactattaccccctctggcaaaacttcttttgcaaaagcctctcgctattttggtttttatcgtcgtctggtaaacgagggttatgatagtgttgctcttactatgcctcgtaattccttttggcgttatgtatctgcattagttgaatgtggtattcctaaatctcaactgatgaatctttctacctgtaataatgttgttccgttagttcgttttattaacgtagatttttcttcccaacgtcctgactggtataatgagccagttcttaaaatcgcataaggtaattcacaatgattaaagttgaaattaaaccatctcaagcccaatttactactcgttctggtgtttctcgtcagggcaagccttattcactgaatgagcagctttgttacgttgatttgggtaatgaatatccggttcttgtcaagattactcttgatgaaggtcagccagcctatgcgcctggtctgtacaccgttcatctgtcctctttcaaagttggtcagttcggttcccttatgattgaccgtctgcgcctcgttccggctaagtaacatggagcaggtcgcggatttcgacacaatttatcaggcgatgatacaaatctccgttgtactttgtttcgcgcttggtataatcgctgggggtcaaagatgagtgttttagtgtattctttcgcctctttcgttttaggttggtgccttcgtagtggcattacgtattttacccgtttaatggaaacttcctcatgaaaaagtctttagtcctcaaagcctctgtagccgttgctaccctcgttccgatgctgtctttcgctgctgagggtgacgatcccgcaaaagcggcctttaactccctgcaagcctcagcgaccgaatatatcggttatgcgtgggcgatggttgttgtcattgtcggcgcaactatcggtatcaagctgtttaagaaattcacctcgaaagcaagctgataaaccgatacaattaaaggctccttttggagcctttttttttggagattttcaacgtgaaaaaattattattcgcaattcctttagttgttcctttctattctcactccgcttgtgattgtaggggggattgtttttgtgaaactgttgaaagttgtttagcaaaaccccatacagaaaattcatttactaacgtctggaaagacgacaaaactttagatcgttacgctaactatgagggttgtctgtggaatgctacaggcgttgtagtttgtactggtgacgaaactcagtgttacggtacatgggttcctattgggcttgctatccctgaaaatgagggtggtggctctgagggtggcggttctgagggtggcggttctgagggtggcggtactaaacctcctgagtacggtgatacacctattccgggctatacttatatcaaccctctcgacggcacttatccgcctggtactgagcaaaaccccgctaatcctaatccttctcttgaggagtctcagcctcttaatactttcatgtttcagaataataggttccgaaataggcagggggcattaactgtttatacgggcactgttactcaaggcactgaccccgttaaaacttattaccagtacactcctgtatcatcaaaagccatgtatgacgcttactggaacggtaaattcagagactgcgctttccattctggctttaatgaggatccattcgtttgtgaatatcaaggccaatcgtctgacctgcctcaacctcctgtcaatgctggcggcggctctggtggtggttctggtggcggctctgagggtggtggctctgagggtggcggttctgagggtggcggctctgagggaggcggttccggtggtggctctggttccggtgattttgattatgaaaagatggcaaacgctaataagggggctatgaccgaaaatgccgatgaaaacgcgctacagtctgacgctaaaggcaaacttgattctgtcgctactgattacggtgctgctatcgatggtttcattggtgacgtttccggccttgctaatggtaatggtgctactggtgattttgctggctctaattcccaaatggctcaagtcggtgacggtgataattcacctttaatgaataatttccgtcaatatttaccttccctccctcaatcggttgaatgtcgcccttttgtctttagcgctggtaaaccatatgaattttctattgattgtgacaaaataaacttattccgtggtgtctttgcgtttcttttatatgttgccacctttatgtatgtattttctacgtttgctaacatactgcgtaataaggagtcttaatcatgccagttcttttgggtattccgttattattgcgtttcctcggtttccttctggtaactttgttcggctatctgcttacttttcttaaaaagggcttcggtaagatagctattgctatttcattgtttcttgctcttattattgggcttaactcaattcttgtgggttatctctctgatattagcgctcaattaccctctgactttgttcagggtgttcagttaattctcccgtctaatgcgcttccctgtttttatgttattctctctgtaaaggctgctattttcatttttgacgttaaacaaaaaatcgtttcttatttggattgggataaataatatggctgtttattttgtaactggcaaattaggctctggaaagacgctcgttagcgttggtaagattcaggataaaattgtagctgggtgcaaaatagcaactaatcttgatttaaggcttcaaaacctcccgcaagtcgggaggttcgctaaaacgcctcgcgttcttagaataccggataagccttctatatctgatttgcttgctattgggcgcggtaatgattcctacgatgaaaataaaaacggcttgcttgttctcgatgagtgcggtacttggtttaatacccgttcttggaatgataaggaaagacagccgattattgattggtttctacatgctcgtaaattaggatgggatattatttttcttgttcaggacttatctattgttgataaacaggcgcgttctgcattagctgaacatgttgtttattgtcgtcgtctggacagaattactttaccttttgtcggtactttatattctcttattactggctcgaaaatgcctctgcctaaattacatgttggcgttgttaaatatggcgattctcaattaagccctactgttgagcgttggctttatactggtaagaatttgtataacgcatatgatactaaacaggctttttctagtaattatgattccggtgtttattcttatttaacgccttatttatcacacggtcggtatttcaaaccattaaatttaggtcagaagatgaaattaactaaaatatatttgaaaaagttttctcgcgttctttgtcttgcgattggatttgcatcagcatttacatatagttatataacccaacctaagccggaggttaaaaaggtagtctctcagacctatgattttgataaattcactattgactcttctcagcgtcttaatctaagctatcgctatgttttcaaggattctaagggaaaattaattaatagcgacgatttacagaagcaaggttattcactcacatatattgatttatgtactgtttccattaaaaaaggtaattcaaatgaaattgttaaatgtaattaattttgttttcttgatgtttgtttcatcatcttcttttgctcaggtaattgaaatgaataattcgcctctgcgcgattttgtaacttggtattcaaagcaatcaggcgaatccgttattgtttctcccgatgtaaaaggtactgttactgtatattcatctgacgttaaacctgaaaatctacgcaatttctttatttctgttttacgtgctaataattttgatatggttggttcaattccttccataattcagaagtataatccaaacaatcaggattatattgatgaattgccatcatctgataatcaggaatatgatgataattccgctccttctggtggtttctttgttccgcaaaatgataatgttactcaaacttttaaaattaataacgttcgggcaaaggatttaatacgagttgtcgaattgtttgtaaagtctaatacttctaaatcctcaaatgtattatctattgacggctctaatctattagttgttagtgcacctaaagatattttagataaccttcctcaattcctttctactgttgatttgccaactgaccagatattgattgagggtttgatatttgaggttcagcaaggtgatgctttagatttttcatttgctgctggctctcagcgtggcactgttgcaggcggtgttaatactgaccgcctcacctctgttttatcttctgctggtggttcgttcggtatttttaatggcgatgttttagggctatcagttcgcgcattaaagactaatagccattcaaaaatattgtctgtgccacgtattcttacgctttcaggtcagaagggttctatctctgttggccagaatgtcccttttattactggtcgtgtgactggtgaatctgccaatgtaaataatccatttcagacgattgagcgtcaaaatgtaggtatttccatgagcgtttttcctgttgcaatggctggcggtaatattgttctggatattaccagcaaggccgatagtttgagttcttctactcaggcaagtgatgttattactaatcaaagaagtattgctacaacggttaatttgcgtgatggacagactcttttactcggtggcctcactgattataaaaacacttctcaagattctggcgtaccgttcctgtctaaaatccctttaatcggcctcctgtttagctcccgctctgattccaacgaggaaagcacgttatacgtgctcgtcaaagcaaccatagtacgcgccctgtagcggcgcattaagcgcggcgggtgtggtggttacgcgcagcgtgaccgctacacttgccagcgccctagcgcccgctcctttcgctttcttcccttcctttctcgccacgttcgccggctttccccgtcaagctctaaatcgggggctccctttagggttccgatttagtgctttacggcacctcgaccccaaaaaacttgatttgggtgatggttcacgtagtgggccatcgccctgatagacggtttttcgccctttgacgttggagtccacgttctttaatagtggactcttgttccaaactggaacaacactcaaccctatctcgggacggatcgcttcatgtggcaggagaaaaaaggctgcaccggtgcgtcagcagaatatgtgatacaggatatattccgcttcctcgctcactgactcgctacgctcggtcgttcgactgcggcgagcggaaatggcttacgaacggggcggagatttcctggaagatgccaggaagatacttaacagggaagtgagagggccgcggcaaagccgtttttccataggctccgcccccctgacaagcatcacgaaatctgacgctcaaatcagtggtggcgaaacccgacaggactataaagataccaggcgtttccccctggcggctccctcgtgcgctctcctgttcctgcctttcggtttaccggtgtcattccgctgttatggccgcgtttgtctcattccacgcctgacactcagttccgggtaggcagttcgctccaagctggactgtatgcacgaaccccccgttcagtccgaccgctgcgccttatccggtaactatcgtcttgagtccaacccggaaagacatgcaaaagcaccactggcagcagccactggtaattgatttagaggagttagtcttgaagtcatgcgccggttaaggctaaactgaaaggacaagttttggtgactgcgctcctccaagccagttacctcggttcaaagagttggtagctcagagaaccttcgaaaaaccgccctgcaaggcggttttttcgttttcagagcaagagattacgcgcagaccaaaacgatctcaagaagatcatcttattaaggggtctgacgctcagtggaacgaaaactcacgttaagggattttggtcatgagattatcaaaaaggatcttcacctagatccttttaaattaaaaatgaagttttaaatcaatctaaagtatatatgagtaaacttggtctgacagttaccaatgcttaatcagtgaggcacctatctcagcgatctgtctatttcgttcatccatagttgcctgactccccgtcgtgtagataactacgatacgggagggcttaccatctggccccagtgctgcaatgataccgcgagacccacgctcaccggctccagatttatcagcaataaaccagccagccgattcgagctcgccccggggatcgaccagttggtgattttgaacttttgctttgccacggaacggtctgcgttgtcgggaagatgcgtgatctgatccttcaactcagcaaaagttcgatttattcaacaaagccgccgtcccgtcaagtcagcgtaatgctctgccagtgttacaaccaattaaccaattctgattagaaaaactcatcgagcatcaaatgaaactgcaatttattcatatcaggattatcaataccatatttttgaaaaagccgtttctgtaatgaaggagaaaactcaccgaggcagttccataggatggcaagatcctggtatcggtctgcgattccgactcgtccaacatcaatacaacctattaatttcccctcgtcaaaaataaggttatcaagtgagaaatcaccatgagtgacgactgaatccggtgagaatggcaaaagcttatgcatttctttccagacttgttcaacaggccagccattacgctcgtcatcaaaatcactcgcatcaaccaaaccgttattcattcgtgattgcgcctgagcgagacgaaatacgcgatcgctgttaaaaggacaattacaaacaggaatcgaatgcaaccggcgcaggaacactgccagcgcatcaacaatattttcacctgaatcaggatattcttctaatacctggaatgctgttttcccggggatcgcagtggtgagtaaccatgcatcatcaggagtacggataaaatgcttgatggtcggaagaggcataaattccgtcagccagtttagtctgaccatctcatctgtaacatcattggcaacgctacctttgccatgtttcagaaacaactctggcgcatcgggcttcccatacaatcgatagattgtcgcacctgattgcccgacattatcgcgagcccatttatacccatataaatcagcatccatgttggaatttaatcgcggcctcgagcaagacgtttcccgttgaatatggctcataacaccccttgtattactgtttatgtaagcagacagttttattgttcatgatgatatatttttatcttgtgcaatgtaacatcagagattttgagacacaacgtggctttccccccccccccctgcaggtctcgggctattcttttgatttataagggattttgccgatttcggcctattggttaaaaaatgagctgatttaacaaaaatttaacgcgaattttaacaaaatattaacgtttacaatttaaatatttgcttatacaatcttcctgtttttggggcttttctgattatcaaccggggtacatatgattgacatgctagttttacgattaccgttcatcgattctcttgtttgctccagactctcaggcaatgacctgatagcctttgtagacctctcaaaaatagctaccctctccggcatgaatttatcagctagaacggttgaatatcatattgatggtgatttgactgtctccggcctttctcacccttttgaatctttacctacacattactcaggcattgcatttaaaatatatgagggttctaaaaatttttatccttgcgttgaaataaaggcttctcccgcaaaagtattacagggtcataatgtttttggtacaaccgatttagctttatgctctgaggctttattgcttaattttgctaattctttgccttgcctgtatgatttattggatgtt

SEQ ID NO: 11 - DNA, 8669 bp, unidentified
  source 1..8669: mol_type = unassigned DNA; note = The nucleic acid sequence of a preferred embodiment of a second vector (i.e.a helper phage without a RGD sequence)
aacgctactactattagtagaattgatgccaccttttcagctcgcgccccaaatgaaaatatagctaaacaggttattgaccatttgcgaaatgtatctaatggtcaaactaaatctactcgttcgcagaattgggaatcaactgttacatggaatgaaacttccagacaccgtactttagttgcatatttaaaacatgttgagctacagcaccagattcagcaattaagctctaagccatccgcaaaaatgacctcttatcaaaaggagcaattaaaggtactctctaatcctgacctgttggagtttgcttccggtctggttcgctttgaagctcgaattaaaacgcgatatttgaagtctttcgggcttcctcttaatctttttgatgcaatccgctttgcttctgactataatagtcagggtaaagacctgatttttgatttatggtcattctcgttttctgaactgtttaaagcatttgagggggattcaatgaatatttatgacgattccgcagtattggacgctatccagtctaaacattttactattaccccctctggcaaaacttcttttgcaaaagcctctcgctattttggtttttatcgtcgtctggtaaacgagggttatgatagtgttgctcttactatgcctcgtaattccttttggcgttatgtatctgcattagttgaatgtggtattcctaaatctcaactgatgaatctttctacctgtaataatgttgttccgttagttcgttttattaacgtagatttttcttcccaacgtcctgactggtataatgagccagttcttaaaatcgcataaggtaattcacaatgattaaagttgaaattaaaccatctcaagcccaatttactactcgttctggtgtttctcgtcagggcaagccttattcactgaatgagcagctttgttacgttgatttgggtaatgaatatccggttcttgtcaagattactcttgatgaaggtcagccagcctatgcgcctggtctgtacaccgttcatctgtcctctttcaaagttggtcagttcggttcccttatgattgaccgtctgcgcctcgttccggctaagtaacatggagcaggtcgcggatttcgacacaatttatcaggcgatgatacaaatctccgttgtactttgtttcgcgcttggtataatcgctgggggtcaaagatgagtgttttagtgtattctttcgcctctttcgttttaggttggtgccttcgtagtggcattacgtattttacccgtttaatggaaacttcctcatgaaaaagtctttagtcctcaaagcctctgtagccgttgctaccctcgttccgatgctgtctttcgctgctgagggtgacgatcccgcaaaagcggcctttaactccctgcaagcctcagcgaccgaatatatcggttatgcgtgggcgatggttgttgtcattgtcggcgcaactatcggtatcaagctgtttaagaaattcacctcgaaagcaagctgataaaccgatacaattaaaggctccttttggagcctttttttttggagattttcaacgtgaaaaaattattattcgcaattcctttagttgttcctttctattctcactccgctgaaactgttgaaagttgtttagcaaaaccccatacagaaaattcatttactaacgtctggaaagacgacaaaactttagatcgttacgctaactatgagggttgtctgtggaatgctacaggcgttgtagtttgtactggtgacgaaactcagtgttacggtacatgggttcctattgggcttgctatccctgaaaatgagggtggtggctctgagggtggcggttctgagggtggcggttctgagggtggcggtactaaacctcctgagtacggtgatacacctattccgggctatacttatatcaaccctctcgacggcacttatccgcctggtactgagcaaaaccccgctaatcctaatccttctcttgaggagtctcagcctcttaatactttcatgtttcagaataataggttccgaaataggcagggggcattaactgtttatacgggcactgttactcaaggcactgaccccgttaaaacttattaccagtacactcctgtatcatcaaaagccatgtatgacgcttactggaacggtaaattcagagactgcgctttccattctggctttaatgaggatccattcgtttgtgaatatcaaggccaatcgtctgacctgcctcaacctcctgtcaatgctggcggcggctctggtggtggttctggtggcggctctgagggtggtggctctgagggtggcggttctgagggtggcggctctgagggaggcggttccggtggtggctctggttccggtgattttgattatgaaaagatggcaaacgctaataagggggctatgaccgaaaatgccgatgaaaacgcgctacagtctgacgctaaaggcaaacttgattctgtcgctactgattacggtgctgctatcgatggtttcattggtgacgtttccggccttgctaatggtaatggtgctactggtgattttgctggctctaattcccaaatggctcaagtcggtgacggtgataattcacctttaatgaataatttccgtcaatatttaccttccctccctcaatcggttgaatgtcgcccttttgtctttagcgctggtaaaccatatgaattttctattgattgtgacaaaataaacttattccgtggtgtctttgcgtttcttttatatgttgccacctttatgtatgtattttctacgtttgctaacatactgcgtaataaggagtcttaatcatgccagttcttttgggtattccgttattattgcgtttcctcggtttccttctggtaactttgttcggctatctgcttacttttcttaaaaagggcttcggtaagatagctattgctatttcattgtttcttgctcttattattgggcttaactcaattcttgtgggttatctctctgatattagcgctcaattaccctctgactttgttcagggtgttcagttaattctcccgtctaatgcgcttccctgtttttatgttattctctctgtaaaggctgctattttcatttttgacgttaaacaaaaaatcgtttcttatttggattgggataaataatatggctgtttattttgtaactggcaaattaggctctggaaagacgctcgttagcgttggtaagattcaggataaaattgtagctgggtgcaaaatagcaactaatcttgatttaaggcttcaaaacctcccgcaagtcgggaggttcgctaaaacgcctcgcgttcttagaataccggataagccttctatatctgatttgcttgctattgggcgcggtaatgattcctacgatgaaaataaaaacggcttgcttgttctcgatgagtgcggtacttggtttaatacccgttcttggaatgataaggaaagacagccgattattgattggtttctacatgctcgtaaattaggatgggatattatttttcttgttcaggacttatctattgttgataaacaggcgcgttctgcattagctgaacatgttgtttattgtcgtcgtctggacagaattactttaccttttgtcggtactttatattctcttattactggctcgaaaatgcctctgcctaaattacatgttggcgttgttaaatatggcgattctcaattaagccctactgttgagcgttggctttatactggtaagaatttgtataacgcatatgatactaaacaggctttttctagtaattatgattccggtgtttattcttatttaacgccttatttatcacacggtcggtatttcaaaccattaaatttaggtcagaagatgaaattaactaaaatatatttgaaaaagttttctcgcgttctttgtcttgcgattggatttgcatcagcatttacatatagttatataacccaacctaagccggaggttaaaaaggtagtctctcagacctatgattttgataaattcactattgactcttctcagcgtcttaatctaagctatcgctatgttttcaaggattctaagggaaaattaattaatagcgacgatttacagaagcaaggttattcactcacatatattgatttatgtactgtttccattaaaaaaggtaattcaaatgaaattgttaaatgtaattaattttgttttcttgatgtttgtttcatcatcttcttttgctcaggtaattgaaatgaataattcgcctctgcgcgattttgtaacttggtattcaaagcaatcaggcgaatccgttattgtttctcccgatgtaaaaggtactgttactgtatattcatctgacgttaaacctgaaaatctacgcaatttctttatttctgttttacgtgctaataattttgatatggttggttcaattccttccataattcagaagtataatccaaacaatcaggattatattgatgaattgccatcatctgataatcaggaatatgatgataattccgctccttctggtggtttctttgttccgcaaaatgataatgttactcaaacttttaaaattaataacgttcgggcaaaggatttaatacgagttgtcgaattgtttgtaaagtctaatacttctaaatcctcaaatgtattatctattgacggctctaatctattagttgttagtgcacctaaagatattttagataaccttcctcaattcctttctactgttgatttgccaactgaccagatattgattgagggtttgatatttgaggttcagcaaggtgatgctttagatttttcatttgctgctggctctcagcgtggcactgttgcaggcggtgttaatactgaccgcctcacctctgttttatcttctgctggtggttcgttcggtatttttaatggcgatgttttagggctatcagttcgcgcattaaagactaatagccattcaaaaatattgtctgtgccacgtattcttacgctttcaggtcagaagggttctatctctgttggccagaatgtcccttttattactggtcgtgtgactggtgaatctgccaatgtaaataatccatttcagacgattgagcgtcaaaatgtaggtatttccatgagcgtttttcctgttgcaatggctggcggtaatattgttctggatattaccagcaaggccgatagtttgagttcttctactcaggcaagtgatgttattactaatcaaagaagtattgctacaacggttaatttgcgtgatggacagactcttttactcggtggcctcactgattataaaaacacttctcaagattctggcgtaccgttcctgtctaaaatccctttaatcggcctcctgtttagctcccgctctgattccaacgaggaaagcacgttatacgtgctcgtcaaagcaaccatagtacgcgccctgtagcggcgcattaagcgcggcgggtgtggtggttacgcgcagcgtgaccgctacacttgccagcgccctagcgcccgctcctttcgctttcttcccttcctttctcgccacgttcgccggctttccccgtcaagctctaaatcgggggctccctttagggttccgatttagtgctttacggcacctcgaccccaaaaaacttgatttgggtgatggttcacgtagtgggccatcgccctgatagacggtttttcgccctttgacgttggagtccacgttctttaatagtggactcttgttccaaactggaacaacactcaaccctatctcgggacggatcgcttcatgtggcaggagaaaaaaggctgcaccggtgcgtcagcagaatatgtgatacaggatatattccgcttcctcgctcactgactcgctacgctcggtcgttcgactgcggcgagcggaaatggcttacgaacggggcggagatttcctggaagatgccaggaagatacttaacagggaagtgagagggccgcggcaaagccgtttttccataggctccgcccccctgacaagcatcacgaaatctgacgctcaaatcagtggtggcgaaacccgacaggactataaagataccaggcgtttccccctggcggctccctcgtgcgctctcctgttcctgcctttcggtttaccggtgtcattccgctgttatggccgcgtttgtctcattccacgcctgacactcagttccgggtaggcagttcgctccaagctggactgtatgcacgaaccccccgttcagtccgaccgctgcgccttatccggtaactatcgtcttgagtccaacccggaaagacatgcaaaagcaccactggcagcagccactggtaattgatttagaggagttagtcttgaagtcatgcgccggttaaggctaaactgaaaggacaagttttggtgactgcgctcctccaagccagttacctcggttcaaagagttggtagctcagagaaccttcgaaaaaccgccctgcaaggcggttttttcgttttcagagcaagagattacgcgcagaccaaaacgatctcaagaagatcatcttattaaggggtctgacgctcagtggaacgaaaactcacgttaagggattttggtcatgagattatcaaaaaggatcttcacctagatccttttaaattaaaaatgaagttttaaatcaatctaaagtatatatgagtaaacttggtctgacagttaccaatgcttaatcagtgaggcacctatctcagcgatctgtctatttcgttcatccatagttgcctgactccccgtcgtgtagataactacgatacgggagggcttaccatctggccccagtgctgcaatgataccgcgagacccacgctcaccggctccagatttatcagcaataaaccagccagccgattcgagctcgccccggggatcgaccagttggtgattttgaacttttgctttgccacggaacggtctgcgttgtcgggaagatgcgtgatctgatccttcaactcagcaaaagttcgatttattcaacaaagccgccgtcccgtcaagtcagcgtaatgctctgccagtgttacaaccaattaaccaattctgattagaaaaactcatcgagcatcaaatgaaactgcaatttattcatatcaggattatcaataccatatttttgaaaaagccgtttctgtaatgaaggagaaaactcaccgaggcagttccataggatggcaagatcctggtatcggtctgcgattccgactcgtccaacatcaatacaacctattaatttcccctcgtcaaaaataaggttatcaagtgagaaatcaccatgagtgacgactgaatccggtgagaatggcaaaagcttatgcatttctttccagacttgttcaacaggccagccattacgctcgtcatcaaaatcactcgcatcaaccaaaccgttattcattcgtgattgcgcctgagcgagacgaaatacgcgatcgctgttaaaaggacaattacaaacaggaatcgaatgcaaccggcgcaggaacactgccagcgcatcaacaatattttcacctgaatcaggatattcttctaatacctggaatgctgttttcccggggatcgcagtggtgagtaaccatgcatcatcaggagtacggataaaatgcttgatggtcggaagaggcataaattccgtcagccagtttagtctgaccatctcatctgtaacatcattggcaacgctacctttgccatgtttcagaaacaactctggcgcatcgggcttcccatacaatcgatagattgtcgcacctgattgcccgacattatcgcgagcccatttatacccatataaatcagcatccatgttggaatttaatcgcggcctcgagcaagacgtttcccgttgaatatggctcataacaccccttgtattactgtttatgtaagcagacagttttattgttcatgatgatatatttttatcttgtgcaatgtaacatcagagattttgagacacaacgtggctttccccccccccccctgcaggtctcgggctattcttttgatttataagggattttgccgatttcggcctattggttaaaaaatgagctgatttaacaaaaatttaacgcgaattttaacaaaatattaacgtttacaatttaaatatttgcttatacaatcttcctgtttttggggcttttctgattatcaaccggggtacatatgattgacatgctagttttacgattaccgttcatcgattctcttgtttgctccagactctcaggcaatgacctgatagcctttgtagacctctcaaaaatagctaccctctccggcatgaatttatcagctagaacggttgaatatcatattgatggtgatttgactgtctccggcctttctcacccttttgaatctttacctacacattactcaggcattgcatttaaaatatatgagggttctaaaaatttttatccttgcgttgaaataaaggcttctcccgcaaaagtattacagggtcataatgtttttggtacaaccgatttagctttatgctctgaggctttattgcttaattttgctaattctttgccttgcctgtatgatttattggatgtt

SEQ ID NO: 12 - DNA, 58 bp, synthetic construct
  source 1..58: mol_type = other DNA; note = A nucleic acid sequence comprising a section of a genome of a helper phage comprising a RGD4C targeting peptide in a pIII minor coat protein
tattctcactccgcttgtgattgtaggggggattgtttttgtgaaactgttgaaagtt

SEQ ID NO: 13 - protein, 19 aa, synthetic construct
  SOURCE 1..19: NOTE = An amino acid sequence comprising a section of a genome of a helper phage comprising a RGD4C targeting peptide in a pIII minor coat protein
YSHSACDCRGDCFCETVES